European Patent Specification EP 4 087 875 B1, published August 28, 2024. Title: TREATMENT OF PEMPHIGUS VULGARIS. Applicant: argenx BVBA. The sequence listing filed with the application follows.

SEQUENCE LISTING (7 sequences)

SEQ ID NO: 1 - protein, 226 aa, Artificial sequence
  Synthetic polypeptide
DKTHTCPPCPAPELLGGPSVFLFPPKPKDTLYITREPEVTCVVVDVSHEDPEVKFNWYVDGVEVHNAKTKPREEQYNSTYRVVSVLTVLHQDWLNGKEYKCKVSNKALPAPIEKTISKAKGQPREPQVYTLPPSRDELTKNQVSLTCLVKGFYPSDIAVEWESNGQPENNYKTTPPVLDSDGSFFLYSKLTVDKSRWQQGNVFSCSVMHEALKFHYTQKSLSLSPG

SEQ ID NO: 2 - protein, 227 aa, Artificial sequence
  Synthetic polypeptide
DKTHTCPPCPAPELLGGPSVFLFPPKPKDTLYITREPEVTCVVVDVSHEDPEVKFNWYVDGVEVHNAKTKPREEQYNSTYRVVSVLTVLHQDWLNGKEYKCKVSNKALPAPIEKTISKAKGQPREPQVYTLPPSRDELTKNQVSLTCLVKGFYPSDIAVEWESNGQPENNYKTTPPVLDSDGSFFLYSKLTVDKSRWQQGNVFSCSVMHEALKFHYTQKSLSLSPGK

SEQ ID NO: 3 - protein, 221 aa, Artificial sequence
  Synthetic polypeptide
CPPCPAPELLGGPSVFLFPPKPKDTLYITREPEVTCVVVDVSHEDPEVKFNWYVDGVEVHNAKTKPREEQYNSTYRVVSVLTVLHQDWLNGKEYKCKVSNKALPAPIEKTISKAKGQPREPQVYTLPPSRDELTKNQVSLTCLVKGFYPSDIAVEWESNGQPENNYKTTPPVLDSDGSFFLYSKLTVDKSRWQQGNVFSCSVMHEALKFHYTQKSLSLSPG

SEQ ID NO: 4 - protein, 216 aa, Artificial sequence
  Synthetic polypeptide
QSALTQPASVSGSPGQSITISCTGTGSDVGSYNLVSWYQQHPGKAPKLMIYGDSERPSGVSNRFSGSKSGNTASLTISGLQAEDEADYYCSSYAGSGIYVFGTGTKVTVLGQPKAAPSVTLFPPSSEELQANKATLVCLISDFYPGAVTVAWKADSSPVKAGVETTTPSKQSNNKYAASSYLSLTPEQWKSHKSYSCQVTHEGSTVEKTVAPTECS

SEQ ID NO: 5 - protein, 445 aa, Artificial sequence
  Synthetic polypeptide
EVQLLESGGGLVQPGGSLRLSCAASGFTFSTYAMGWVRQAPGKGLEWVSSIGASGSQTRYADSVKGRFTISRDNSKNTLYLQMNSLRAEDTAVYYCARLAIGDSYWGQGTMVTVSSASTKGPSVFPLAPSSKSTSGGTAALGCLVKDYFPEPVTVSWNSGALTSGVHTFPAVLQSSGLYSLSSVVTVPSSSLGTQTYICNVNHKPSNTKVDKKVEPKSCDKTHTCPPCPAPELLGGPSVFLFPPKPKDTLMISRTPEVTCVVVDVSHEDPEVKFNWYVDGVEVHNAKTKPREEQYASTYRVVSVLTVLHQDWLNGKEYKCKVSNKALPAPIEKTISKAKGQPREPQVYTLPPSREEMTKNQVSLTCLVKGFYPSDIAVEWESNGQPENNYKTTPPVLDSDGSFFLYSKLTVDKSRWQQGNVFSCSVMHEALHNHYTQKSLSLSPG

SEQ ID NO: 6 - protein, 219 aa, Artificial sequence
  Synthetic polypeptide
DIQMTQSPSSLSASVGDRVTITCKSSQSLVGASGKTYLYWLFQKPGKAPKRLIYLVSTLDSGIPSRFSGSGSGTEFTLTISSLQPEDFATYYCLQGTHFPHTFGQGTKLEIKRTVAAPSVFIFPPSDEQLKSGTASVVCLLNNFYPREAKVQWKVDNALQSGNSQESVTEQDSKDSTYSLSSTLTLSKADYEKHKVYACEVTHQGLSSPVTKSFNRGEC

SEQ ID NO: 7 - protein, 444 aa, Artificial sequence
  Synthetic polypeptide
EVPLVESGGGLVQPGGSLRLSCAVSGFTFSNYGMVWVRQAPGKGLEWVAYIDSDGDNTYYRDSVKGRFTISRDNAKSSLYLQMNSLRAEDTAVYYCTTGIVRPFLYWGQGTLVTVSSASTKGPSVFPLAPCSRSTSESTAALGCLVKDYFPEPVTVSWNSGALTSGVHTFPAVLQSSGLYSLSSVVTVPSSSLGTKTYTCNVDHKPSNTKVDKRVESKYGPPCPPCPAPEFLGGPSVFLFPPKPKDTLMISRTPEVTCVVVDVSQEDPEVQFNWYVDGVEVHNAKTKPREEQFNSTYRVVSVLTVLHQDWLNGKEYKCKVSNKGLPSSIEKTISKAKGQPREPQVYTLPPSQEEMTKNQVSLTCLVKGFYPSDIAVEWESNGQPENNYKTTPPVLDSDGSFFLYSRLTVDKSRWQEGNVFSCSVMHEALHNHYTQKSLSLSLGK